European Patent Specification EP 3 845 237 B1, published January 7, 2026. Title: Use of novel recombinant protein Ablysin killing pathogenic multidrug resistant bacteria. Applicant: KYUNGPOOK NATIONAL UNIVERSITY INDUSTRY-ACADEMIC COOPERATION FOUNDATION. The sequence listing filed with the application follows.

SEQUENCE LISTING (2 sequences)

SEQ ID NO: 1 - protein, 252 aa, Acinetobacter baumannii
MTKLAKTFSAPRYNTLIGIVLACVMGVLTYFGLFYQQKAIAQDYPVQGFDVSHHQENINWKKISPKKFQFVYLKATEGGDYKDPKFQENWLKAREHGFHVGAYHFYRLCRDGKTQAENFISTVPNKADALPPVIDLEYDSNCINSHTKEQLLKEIGIMHDSLKHHYGKQPIFYISKTFYHIVLIGSFPHTPLWVRDYEGKPELKDKRKWLFWQHSNQGKIEGITKPVDLNVYEGSVKEWHQFLQQQGIVKAQ

SEQ ID NO: 2 - DNA, 759 bp, Acinetobacter baumannii
atgaccaagctggcaaaaaccttttctgcaccacgctacaatacccttattgggattgttttagcttgtgttatgggggttctcacctacttcggtctgttctaccagcaaaaagctattgctcaagattacccagttcaaggctttgatgtctctcaccatcaagaaaatattaactggaaaaaaatatcacccaaaaaattccagttcgtctatttaaaagcgactgaaggcggtgattataaagatccaaaatttcaagaaaactggttaaaagcacgcgaacatggctttcatgtcggggcttatcatttttatcgtttatgtcgtgatggcaaaacacaagctgaaaattttatttcaaccgtacccaacaaagctgatgcccttcctcccgttattgatctggaatatgacagcaactgtattaattctcataccaaagaacaattacttaaagaaataggcatcatgcatgacagcttaaagcatcattatggtaaacagcctatcttttatatttccaaaactttttaccatattgtattaataggtagtttccctcatacacctctttgggtcagagattacgaagggaaacctgagctgaaagacaagcgaaaatggctcttttggcagcatagtaatcaaggtaaaattgaaggcatcaccaagccagtagacttaaatgtttatgaaggttcagtcaaagaatggcaccaatttttacagcagcaaggcatcgtgaaagcacaatga